European Patent Application EP 4 455 162 A1, published October 30, 2024. Title: Fusion proteins composed of an antibody and an interleukin 2 no alpha mutein. Applicant: CENTRO DE INMUNOLOGIA MOLECULAR. Application CU 2021-0104, filed December 21, 2021. The sequence listing filed with the application follows.

SEQUENCE LISTING (45 sequences)

SEQ ID NO: 1 - protein, 106 aa, synthetic construct [sequence omitted]

SEQ ID NO: 2 - protein, 121 aa, synthetic construct [sequence omitted]

SEQ ID NO: 3 - protein, 107 aa, synthetic construct
DLVLTQSPATLSVTPGDSVSFSCRASQSISNNLHWYQQKPGQSPRLLIKYASQSISGVPSRFSGSGSGTDFTLSIISVETEDFGMYFCQQSNRWPLTFGAGTKLELK

SEQ ID NO: 4 - protein, 125 aa, synthetic construct
QVQLVQSGAEVVKPGASMKMSCRASGYSFTSYWIHWLKQRPDQGLEWVGYIDPATAYTESNQKFKDKAILTADRSSNTAFMYLNSLTSEDSAVYYCARESPRLRRGIYYYAMDYWGQGTTVTVSS

SEQ ID NO: 5 - protein, 113 aa, synthetic construct
DIQMTQSPSSLSASVGDRVTITCRSSQNIVHSNGNTYLDWYQQTPGKAPKLLIYKVSNRFSGVPSRFSGSGSGTDFTFTISSLQPEDIATYYCFQYSHVPWTFGQGTKLQITR

SEQ ID NO: 6 - protein, 123 aa, synthetic construct [sequence omitted]

SEQ ID NO: 7 - protein, 107 aa, synthetic construct
DLVLTQSPATLSVTPGDSVSFSCRASQSISNNLHWYQQRTHESPRLLIKYASQSISGIPSRFSGSGSGTDFTLSIISVETEDFGMYFCQQSNRWPLTFGAGTKLELK

SEQ ID NO: 8 - protein, 125 aa, synthetic construct
QVQLQQSGNELAKPGASMKMSCRASGYSFTSYWIHWLKQRPDQGLEWIGYIDPATAYTESNQKFKDKAILTADRSSNTAFMYLNSLTSEDSAVYYCARESPRLRRGIYYYAMDYWGQGTTVTVSS

SEQ ID NO: 9 - protein, 106 aa, synthetic construct
TVAAPSVFIFPPSDEQLKSGTASVVCLLNNFYPREAKVQWKVDNALQSGNSQESVTEQDSKDSTYSLSSTLTLSKADYEKHKVYACEVTHQGLSSPVTKSFNRGEC

SEQ ID NO: 10 - protein, 106 aa, synthetic construct
GQPKAAPSVTLFPPSSEELQANKATLVCLISDFYPGAVTVAWKADSSPVKAGVETTTPSKQSNNKYAASSYLSLTPEQWKSHRSYSCQVTHEGSTVEKTVAPTECS

SEQ ID NO: 11 - protein, 330 aa, synthetic construct
ASTKGPSVFPLAPSSKSTSGGTAALGCLVKDYFPEPVTVSWNSGALTSGVHTFPAVLQSSGLYSLSSVVTVPSSSLGTQTYICNVNHKPSNTKVDKKVEPKSCDKTHTCPPCPAPELLGGPSVFLFPPKPKDTLMISRTPEVTCVVVDVSHEDPEVKFNWYVDGVEVHNAKTKPREEQYNSTYRVVSVLTVLHQDWLNGKEYKCKVSNKALPAPIEKTISKAKGQPREPQVYTLPPSREEMTKNQVSLTCLVKGFYPSDIAVEWESNGQPENNYKTTPPVLDSDGSFFLYSKLTVDKSRWQQGNVFSCSVMHEALHNHYTQKSLSLSPGK

SEQ ID NO: 12 - protein, 377 aa, synthetic construct
ASTKGPSVFPLAPCSRSTSGGTAALGCLVKDYFPEPVTVSWNSGALTSGVHTFPAVLQSSGLYSLSSVVTVPSSSLGTQTYTCNVNHKPSNTKVDKRVELKTPLGDTTHTCPRCPEPKSCDTPPPCPRCPEPKSCDTPPPCPRCPEPKSCDTPPPCPRCPAPELLGGPSVFLFPPKPKDTLMISRTPEVTCVVVDVSHEDPEVQFKWYVDGVEVHNAKTKPREEQYNSTFRVVSVLTVLHQDWLNGKEYKCKVSNKALPAPIEKTISKTKGQPREPQVYTLPPSREEMTKNQVSLTCLVKGFYPSDIAVEWESSGQPENNYNTTPPMLDSDGSFFLYSKLTVDKSRWQQGNIFSCSVMHEALHNRFTQKSLSLSPGK

SEQ ID NO: 13 - protein, 106 aa, synthetic construct
ADAAPTVSIFPPSSEQLTSGGASVVCFLNNFYPKDINVKWKIDGSERQNGVLNSWTDQDSKDSTYSMSSTLTLTKDEYERHNSYTCEATHKTSTSPIVKSFNRNEC

SEQ ID NO: 14 - protein, 324 aa, synthetic construct
AKTTPPSVYPLAPGSAAQTNSMVTLGCLVKGYFPEPVTVTWNSGSLSSGVHTFPAVLQSDLYTLSSSVTVPSSTWPSETVTCNVAHPASSTKVDKKIVPRDCGCKPCICTVPEVSSVFIFPPKPKDVLTITLTPKVTCVVVDISKDDPEVQFSWFVDDVEVHTAQTQPREEQFNSTFRSVSELPIMHQDWLNGKEFKCRVNSAAFPAPIEKTISKTKGRPKAPQVYTIPPPKEQMAKDKVSLTCMITDFFPEDITVEWQWNGQPAENYKNTQPIMDTDGSYFVYSKLNVQKSNWEAGNTFTCSVLHEGLHNHHTEKSLSHSPGK

SEQ ID NO: 15 - protein, 330 aa, synthetic construct
AKTTAPSVYPLAPVCGDTTGSSVTLGCLVKGYFPEPVTLTWNSGSLSSGVHTFPAVLQSDLYTLSSSVTVTSSTWPSQSITCNVAHPASSTKVDKKIEPRGPTIKPCPPCKCPAPNLLGGPSVFIFPPKIKDVLMISLSPIVTCVVVDVSEDDPDVQISWFVNNVEVHTAQTQTHREDYNSTLRVVSALPIQHQDWMSGKEFKCKVNNKDLPAPIERTISKPKGSVRAPQVYVLPPPEEEMTKKQVTLTCMVTDFMPEDIYVEWTNNGKTELNYKNTEPVLDSDGSYFMYSKLRVEKKNWVERNSYSCSVVHEGLHNHHTTKSFSRTPGK

SEQ ID NO: 16 - protein, 133 aa, synthetic construct
APTSSSTKKTQLQLEHLLLDLQMILNGINNYKNPKLTKMLTIKFNMPKKATELKHLQCLEELLKPLEVVLNLAQSKNFHLRPRDLISNINVIVLELKGSETTFMCEYADETATIVEFLNRWITFSQSIISTLT

SEQ ID NO: 17 - protein, 133 aa, synthetic construct
APTSSSTKKTQLQLEHLLLDLQMILNGINNYKNPELTKMLTIKFNMPKKATELKHLQCLEELLKPLEVVLNLAQSKNFHLRPRDLISNINVIVLELKGSETTFMCEYADETATIVEFLNRWITFSQSIISTLT

SEQ ID NO: 18 - protein, 133 aa, synthetic construct
APTSSSTKKTQLQLEHLLLDLQMILNGINNYKNPDLTKMLTIKFNMPKKATELKHLQCLEELLKPLEVVLNLAQSKNFHLRPRDLISNINVIVLELKGSETTFMCEYADETATIVEFLNRWITFSQSIISTLT

SEQ ID NO: 19 - protein, 133 aa, synthetic construct
APTSSSTKKTQLQLEHLLLDLQMILNGINNYKNPQLTKMLTIKFNMPKKATELKHLQCLEELLKPLEVVLNLAQSKNFHLRPRDLISNINVIVLELKGSETTFMCEYADETATIVEFLNRWITFSQSIISTLT

SEQ ID NO: 20 - protein, 133 aa, synthetic construct
APTSSSTKKTQLQLEHLLLDLQMILNGINNYKNPKLTKMLTQKFEMPKKATELKHLQCLEEELKPLEVVLNLAQSKNFHLRPRDLISNINVIVLELKGSETTFMCEYADETATIVEFLNRWITFSQSIISTLT

SEQ ID NO: 21 - protein, 133 aa, synthetic construct
APTSSSTKKTQLQLEHLLLDLQMILNGINNYKNPELTKMLTQKFEMPKKATELKHLQCLEEELKPLEVVLNLAQSKNFHLRPRDLISNINVIVLELKGSETTFMCEYADETATIVEFLNRWITFSQSIISTLT

SEQ ID NO: 22 - protein, 133 aa, synthetic construct
APTSSSTKKTQLQLEHLLLDLQMILNGINNYKNPDLTKMLTQKFEMPKKATELKHLQCLEEELKPLEVVLNLAQSKNFHLRPRDLISNINVIVLELKGSETTFMCEYADETATIVEFLNRWITFSQSIISTLT

SEQ ID NO: 23 - protein, 133 aa, synthetic construct
APTSSSTKKTQLQLEHLLLDLQMILNGINNYKNPQLTKMLTQKFEMPKKATELKHLQCLEEELKPLEVVLNLAQSKNFHLRPRDLISNINVIVLELKGSETTFMCEYADETATIVEFLNRWITFSQSIISTLT

SEQ ID NO: 24 - protein, 133 aa, synthetic construct
APTSSSTKKTQLQLEHLLLDLQMILNGINNYKNPKLTAMLTIKFNMPKKATELKHLQCLEELLKPLEVVLNLAQSKNFHLRPRDLISNINVIVLELKGSETTFMCEYADETATIVEFLNRWITFSQSIISTLT

SEQ ID NO: 25 - protein, 133 aa, synthetic construct
APTSSSTKKTQLQLEHLLLDLQMILNGINNYKNPELTAMLTIKFNMPKKATELKHLQCLEELLKPLEVVLNLAQSKNFHLRPRDLISNINVIVLELKGSETTFMCEYADETATIVEFLNRWITFSQSIISTLT

SEQ ID NO: 26 - protein, 133 aa, synthetic construct
APTSSSTKKTQLQLEHLLLDLQMILNGINNYKNPDLTAMLTIKFNMPKKATELKHLQCLEELLKPLEVVLNLAQSKNFHLRPRDLISNINVIVLELKGSETTFMCEYADETATIVEFLNRWITFSQSIISTLT

SEQ ID NO: 27 - protein, 133 aa, synthetic construct
APTSSSTKKTQLQLEHLLLDLQMILNGINNYKNPQLTAMLTIKFNMPKKATELKHLQCLEELLKPLEVVLNLAQSKNFHLRPRDLISNINVIVLELKGSETTFMCEYADETATIVEFLNRWITFSQSIISTLT

SEQ ID NO: 28 - protein, 133 aa, synthetic construct
APTSSSTKKTQLQLEHLLLDLQMILNGINNYKNPKLTKMLTKKFRMPKKATELKHLQCLEELLKPLEVVLNLAQSKNFHLRPRDLISNINVIVLELKGSETTFMCEYADETATIVEFLNRWITFSQSIISTLT

SEQ ID NO: 29 - protein, 133 aa, synthetic construct
APTSSSTKKTQLQLEHLLLDLQMILNGINNYKNPELTKMLTKKFRMPKKATELKHLQCLEELLKPLEVVLNLAQSKNFHLRPRDLISNINVIVLELKGSETTFMCEYADETATIVEFLNRWITFSQSIISTLT

SEQ ID NO: 30 - protein, 133 aa, synthetic construct
APTSSSTKKTQLQLEHLLLDLQMILNGINNYKNPDLTKMLTKKFRMPKKATELKHLQCLEELLKPLEVVLNLAQSKNFHLRPRDLISNINVIVLELKGSETTFMCEYADETATIVEFLNRWITFSQSIISTLT

SEQ ID NO: 31 - protein, 133 aa, synthetic construct
APTSSSTKKTQLQLEHLLLDLQMILNGINNYKNPQLTKMLTKKFRMPKKATELKHLQCLEELLKPLEVVLNLAQSKNFHLRPRDLISNINVIVLELKGSETTFMCEYADETATIVEFLNRWITFSQSIISTLT

SEQ ID NO: 32 - protein, 133 aa, synthetic construct
APTSSSTKKTQLQLEHLLLDLQMILNGINNYKNPKLTKMLTIKFEMPKKATELKHLQCLEEELKPLEVVLNLAQSKNFHLRPRDLISNINVIVLELKGSETTFMCEYADETATIVEFLNRWITFSQSIISTLT

SEQ ID NO: 33 - protein, 133 aa, synthetic construct
APTSSSTKKTQLQLEHLLLDLQMILNGINNYKNPELTKMLTIKFEMPKKATELKHLQCLEEELKPLEVVLNLAQSKNFHLRPRDLISNINVIVLELKGSETTFMCEYADETATIVEFLNRWITFSQSIISTLT

SEQ ID NO: 34 - protein, 133 aa, synthetic construct
APTSSSTKKTQLQLEHLLLDLQMILNGINNYKNPDLTKMLTIKFEMPKKATELKHLQCLEEELKPLEVVLNLAQSKNFHLRPRDLISNINVIVLELKGSETTFMCEYADETATIVEFLNRWITFSQSIISTLT

SEQ ID NO: 35 - protein, 133 aa, synthetic construct
APTSSSTKKTQLQLEHLLLDLQMILNGINNYKNPQLTKMLTIKFEMPKKATELKHLQCLEEELKPLEVVLNLAQSKNFHLRPRDLISNINVIVLELKGSETTFMCEYADETATIVEFLNRWITFSQSIISTLT

SEQ ID NO: 36 - protein, 133 aa, unidentified
APTSSSTKKTQLQLEHLLLDLQMILNGINNYKNPKLTAMLTAKFAMPKKATELKHLQCLEEALKPLEEVLNLAQSKNFHLRPRDLISNINVIVLELKGSETTFMCEYADETATIVEFLNRWITFSQSIISTLT

SEQ ID NO: 37 - protein, 133 aa, synthetic construct
APTSSSTKKTQLQLEHLLLDLQMILNGINNYKNPELTAMLTAKFAMPKKATELKHLQCLEEALKPLEEVLNLAQSKNFHLRPRDLISNINVIVLELKGSETTFMCEYADETATIVEFLNRWITFSQSIISTLT

SEQ ID NO: 38 - protein, 133 aa, synthetic construct
APTSSSTKKTQLQLEHLLLDLQMILNGINNYKNPDLTAMLTAKFAMPKKATELKHLQCLEEALKPLEEVLNLAQSKNFHLRPRDLISNINVIVLELKGSETTFMCEYADETATIVEFLNRWITFSQSIISTLT

SEQ ID NO: 39 - protein, 133 aa, synthetic construct
APTSSSTKKTQLQLEHLLLDLQMILNGINNYKNPQLTAMLTAKFAMPKKATELKHLQCLEEALKPLEEVLNLAQSKNFHLRPRDLISNINVIVLELKGSETTFMCEYADETATIVEFLNRWITFSQSIISTLT

SEQ ID NO: 40 - protein, 133 aa, synthetic construct
APASSSTKKTQLQLEHLLLDLQMILNGINNYKNPKLTRMLTAKFAMPKKATELKHLQCLEEELKPLEEVLNAAQSKNFHLRPRDLISNINVIVLELKGSETTFMCEYADETATIVEFLNRWITFAESIISTLT

SEQ ID NO: 41 - protein, 133 aa, synthetic construct
APASSSTKKTQLQLEHLLLDLQMILNGINNYKNPELTRMLTAKFAMPKKATELKHLQCLEEELKPLEEVLNAAQSKNFHLRPRDLISNINVIVLELKGSETTFMCEYADETATIVEFLNRWITFAESIISTLT

SEQ ID NO: 42 - protein, 133 aa, synthetic construct
APASSSTKKTQLQLEHLLLDLQMILNGINNYKNPDLTRMLTAKFAMPKKATELKHLQCLEEELKPLEEVLNAAQSKNFHLRPRDLISNINVIVLELKGSETTFMCEYADETATIVEFLNRWITFAESIISTLT

SEQ ID NO: 43 - protein, 133 aa, synthetic construct
APASSSTKKTQLQLEHLLLDLQMILNGINNYKNPQLTRMLTAKFAMPKKATELKHLQCLEEELKPLEEVLNAAQSKNFHLRPRDLISNINVIVLELKGSETTFMCEYADETATIVEFLNRWITFAESIISTLT

SEQ ID NO: 44 - protein, 7 aa, synthetic construct
GGGGSTG

SEQ ID NO: 45 - protein, 5 aa, synthetic construct
GGGGS